European Patent Application EP 4 732 849 A1, published April 29, 2026. Title: Method of improving stability of nucleic acid in blood and improving targeting efficiency. Applicant: Kawasaki Institute of Industrial Promotion. The sequence listing filed with the application follows.

SEQUENCE LISTING (23 sequences)

SEQ ID NO: 1 - RNA, 21 nt, synthetic construct
  source 1..21: mol_type = other RNA
gaagatcaccctccttaaata

SEQ ID NO: 2 - RNA, 23 nt, synthetic construct
  source 1..23: mol_type = other RNA
tatttaaggagggtgatcttctt

SEQ ID NO: 3 - RNA, 21 nt, synthetic construct
  source 1..21: mol_type = other RNA
caggatcatctcaagtcttac

SEQ ID NO: 4 - RNA, 23 nt, synthetic construct
  source 1..23: mol_type = other RNA
gtaagacttgagatgatcctgtt

SEQ ID NO: 5 - protein, 5 aa, synthetic construct
GRGDS

SEQ ID NO: 6 - protein, 5 aa, synthetic construct
  SITE 4: note = D-phe
  REGION 1..5: note = circular
RGFXV

SEQ ID NO: 7 - protein, 5 aa, synthetic construct
  REGION 1..5: note = circular
  SITE 4: note = D-Phe
RGDXK

SEQ ID NO: 8 - protein, 5 aa, synthetic construct
  SITE 4: note = D-Tyr
  REGION 1..5: note = circular
RGDXV

SEQ ID NO: 9 - protein, 5 aa, synthetic construct
  REGION 1..5: note = circular
  SITE 4: note = D-Phe
RGDXY

SEQ ID NO: 10 - protein, 5 aa, synthetic construct
  REGION 1..5: note = circular
  SITE 4: note = D-Tyr
RGDXK

SEQ ID NO: 11 - protein, 4 aa, synthetic construct
REDV

SEQ ID NO: 12 - protein, 5 aa, synthetic construct
YIGSR

SEQ ID NO: 13 - protein, 5 aa, synthetic construct
PDSGR

SEQ ID NO: 14 - protein, 7 aa, synthetic construct
RYVVLPR

SEQ ID NO: 15 - protein, 6 aa, synthetic construct
LGTIPG

SEQ ID NO: 16 - protein, 10 aa, Synthetic construct
RNIAEIIKDI

SEQ ID NO: 17 - protein, 5 aa, synthetic construct
IKVAV

SEQ ID NO: 18 - protein, 4 aa, synthetic construct
DGEA

SEQ ID NO: 19 - protein, 5 aa, synthetic construct
YIGSR

SEQ ID NO: 20 - protein, 5 aa, synthetic construct
PDSGR

SEQ ID NO: 21 - protein, 6 aa, synthetic construct
LGTIPG

SEQ ID NO: 22 - protein, 5 aa, synthetic construct
IKVAV

SEQ ID NO: 23 - protein, 4 aa, synthetic construct
ERGD